European Patent Application EP 4 502 168 A1, published February 5, 2025. Title: Methods for producing lactodiphcotetraose (LDFT). Applicant: KIRIN HOLDINGS KABUSHIKI KAISHA. Application EP 23775120.1, filed March 24, 2023. The sequence listing filed with the application follows.

SEQUENCE LISTING (64 sequences)

SEQ ID NO: 1 - DNA, 954 bp, Bacteroides reticulotermitis and Bacteroides fragilis
  source 1..954: mol_type = genomic DNA
atgaaattgaaagtgaaatttgtagatttttgggatggctttgatgaacattataatactttcgttaatgttctatctgagaaatatgaaatcgaaatttgtgatcatcctgattacttaatatattcgacttttggatataagaacttaaagtacgaaaattgtgttaagatattttatacgggtgaaaatataactccagactttaatctttgtgattatgcgattggctttgatataatggaattcggagatcgctatatgcgcctaccattatatgccttatatggtattgaagagttgcgtaaacctaaagtctttaattcacaggaagctctgaatcgtaagttctgcagcatcgtggttagcaataataaatgggcggacccgattcgtgagacctttttcaaactgctgagcagctacaaaaaggtggacagcggtggccgtgcgtggaacaacatcggtggcccggttgacaacaagctggatttcatcagccagtacaaattcaacattgcgtttgagaacagccgtgtgctgggttacaccaccgaaaagattatggagccgatgcaagtgaacagcattccggtttactggggtaacagattggttgagttggattttaatcctaattcttttattaatgctgcagattacccatctttagaagctttggtagaatatatcgttgagttggacacaaatgatgataaatatctgtcaattttgtcaagaccttggcttaacaaaagtaattatttggattggcaagaaaggctttttagcttctttgagaatgttttcaataaaccattgaatgaacagaaatatttatcaccttatgggtacggtaagctatatagaagaagattaatggaaatgtatattgcgaaaagaaaattgaaaaaatggaaaatggtttgtaacccttgtcgttggtttagatga

SEQ ID NO: 2 - protein, 317 aa, Bacteroides reticulotermitis and Bacteroides fragilis
MKLKVKFVDFWDGFDEHYNTFVNVLSEKYEIEICDHPDYLIYSTFGYKNLKYENCVKIFYTGENITPDFNLCDYAIGFDIMEFGDRYMRLPLYALYGIEELRKPKVFNSQEALNRKFCSIVVSNNKWADPIRETFFKLLSSYKKVDSGGRAWNNIGGPVDNKLDFISQYKFNIAFENSRVLGYTTEKIMEPMQVNSIPVYWGNRLVELDFNPNSFINAADYPSLEALVEYIVELDTNDDKYLSILSRPWLNKSNYLDWQERLFSFFENVFNKPLNEQKYLSPYGYGKLYRRRLMEMYIAKRKLKKWKMVCNPCRWFR

SEQ ID NO: 3 - DNA, 1278 bp, Helicobacter pylori 26695
  source 1..1278: mol_type = genomic DNA
atgttccaacccctattagacgcctttatagaaagcgcttccattgaaaaaatggcctctaaatctccccccccccccctaaaaatcgctgtggcgaattggtggggagatgaagaaattaaagaatttaaaaagagcgttctttattttatcctaagccaacgctacgcaatcaccctccaccaaaaccccaatgaattttcagatctagtttttagcaatcctcttggagcggctagaaagattttatcttatcaaaacactaaacgagtgttttacaccggtgaaaacgaatcacctaatttcaacctctttgattacgccataggctttgatgaattggattttaatgatcgttatttgagaatgcctttgtattatgcccatttgcactataaagccgagcttgttaatgacaccactgcgccctacaaactcaaagacaacagcctttatgctttaaaaaaaccctctcatcattttaaagaaaaccaccctaatttgtgcgcagtagtgaatgatgagagcgatcttttaaaaagagggtttgccagttttgtagcgagcaacgctaacgctcctatgaggaacgctttttatgacgctctaaattccatagagccagttactgggggaggaagtgtgagaaacactttaggctataaggttggaaacaaaagcgagtttttaagccaatacaagttcaatctctgttttgaaaactcgcaaggttatggctatgtaaccgaaaaaatccttgatgcgtattttagccataccattcctatttattgggggagtcccagcgtggcgaaagattttaaccctaaaagttttgtgaatgtgcatgatttcaacaactttgatgaagcgattgattatatcaaatacctgcacacgcacccaaacgcttatttagacatgctctatgaaaaccctttaaacacccttgatgggaaagcttacttttaccaagatttgagttttaaaaaaatcctagatttttttaaaacgattttagaaaacgatacgatttatcacaaattctcaacatctttcatgtgggagtacgatctgcataagccgttagtatccattgatgatttgagggttaattatgatgatttgagggttaattatgaccggcttttacaaaacgcttcgcctttattagaactctctcaaaacaccacttttaaaatctatcgcaaagcttatcaaaaatccttgcctttgttgcgcgcggtgagaaagttggttaaaaaattgggtttgtaa

SEQ ID NO: 4 - protein, 425 aa, Helicobacter pylori 26695
MFQPLLDAFIESASIEKMASKSPPPPLKIAVANWWGDEEIKEFKKSVLYFILSQRYAITLHQNPNEFSDLVFSNPLGAARKILSYQNTKRVFYTGENESPNFNLFDYAIGFDELDFNDRYLRMPLYYAHLHYKAELVNDTTAPYKLKDNSLYALKKPSHHFKENHPNLCAVVNDESDLLKRGFASFVASNANAPMRNAFYDALNSIEPVTGGGSVRNTLGYKVGNKSEFLSQYKFNLCFENSQGYGYVTEKILDAYFSHTIPIYWGSPSVAKDFNPKSFVNVHDFNNFDEAIDYIKYLHTHPNAYLDMLYENPLNTLDGKAYFYQDLSFKKILDFFKTILENDTIYHKFSTSFMWEYDLHKPLVSIDDLRVNYDDLRVNYDRLLQNASPLLELSQNTTFKIYRKAYQKSLPLLRAVRKLVKKLGL

SEQ ID NO: 5 - DNA, 996 bp, Bacteroides fragilis ATCC 25285
  source 1..996: mol_type = genomic DNA
atgtgtgattgcttgtctatcatattgttagtcaaaatgaaaaagatttatttgaaatttgttgatttttgggatggatttgatactatttctaactttattgtggatgctttgtccattcaatacgaagtagtactatctaatgagccagattatttattctattcatgttttggaacgtcacatttagaatatgattgtataaaaatcatgtttataggtgaaaatatagttcctgattttaacgtttgtgattatgccataggttttaattatattgattttggggaccgttacttgaggttgcctttatatgctatatatgatggattttcaaacttgcagaataaaaagattgatgtaaataaagctttagaccgtaaattttgtagtattgttgtttcaaataataaatgggcagatcctattcgtgagactttctttaaattactatctagttataagaaagtagactctggtggaagagcttggaataatataggaggacctgttgataataaattggattttattagccaatataagtttaatattgcttttgaaaatagtagggtactgggatatacaacagaaaaaataatggaacctatgcaggtgaattctattccagtatattggggaaatcctttggttggtaaagattttaatgtggactcctttgtaaatgctcatgattttgattctttagaaagattagttgagtatattatagaattggattcttcaaaggataaatatctggaaatgttggaaaaaccttggcttctcgataagacatatttggattggaaacaattgctgttaaattttattaataatattatgatgaaatcatataaggatgcgaagtatttggttaattatggtcatgctggaaagtatagaaatgaacaacgcttttgggggagatgtgaacgtaaatttaaacttcaaagaattattgaatattattctcaattgtttgatagaaaataa

SEQ ID NO: 6 - protein, 331 aa, Bacteroides fragilis ATCC 25285
MCDCLSIILLVKMKKIYLKFVDFWDGFDTISNFIVDALSIQYEVVLSNEPDYLFYSCFGTSHLEYDCIKIMFIGENIVPDFNVCDYAIGFNYIDFGDRYLRLPLYAIYDGFSNLQNKKIDVNKALDRKFCSIVVSNNKWADPIRETFFKLLSSYKKVDSGGRAWNNIGGPVDNKLDFISQYKFNIAFENSRVLGYTTEKIMEPMQVNSIPVYWGNPLVGKDFNVDSFVNAHDFDSLERLVEYIIELDSSKDKYLEMLEKPWLLDKTYLDWKQLLLNFINNIMMKSYKDAKYLVNYGHAGKYRNEQRFWGRCERKFKLQRIIEYYSQLFDRK

SEQ ID NO: 7 - DNA, 861 bp, Helicobacter mustelae ATCC43772
  source 1..861: mol_type = genomic DNA
atggattttaagattgtgcaagtgcatggaggacttggaaatcagatgtttcaatacgcttttgccaagagtttgcaaacacatctcaatatacccgtgctacttgataccacctggtttgattatggcaatcgggaattgggattgcatctttttcccatcgatttgcaatgtgctagtgcacagcaaattgctgctgcccatatgcaaaacctgccaaggctagtgagaggtgcgctcagacgtatgggtctaggcagagtcagcaaggaaatcgtgtttgaatacatgccagagctgtttgagccaagtcgcattgcttattttcatggctatttccaagatccaagatattttgaagacatctctcccctgattaagcaaacattcaccctgcctcaccccacagagcatgcagagcaatatagccgcaaactctctcagattttggcggcaaaaaatagcgtatttgtgcatataaggcgaggggattatatgagacttggctggcaacttgatatcagctaccaactacgcgccattgcatatatggccaagcgcgtgcaaaatttggagctatttttattttgcgaggatttggaatttgtgcagaatcttgatcttggctatccctttgtggatatgaccacaagggatggggcggcgcattgggatatgatgctgatgcaatcttgcaagcatggcattatcacaaatagtacctatagttggtgggcggcatatttgataaaaaatccagaaaaaatcattattggaccaagccactggatctatggcaatgaaaatatcctttgcaaggattgggtgaagatagaatcccaatttgagacaaaatcttga

SEQ ID NO: 8 - protein, 286 aa, Helicobacter mustelae ATCC43772
MDFKIVQVHGGLGNQMFQYAFAKSLQTHLNIPVLLDTTWFDYGNRELGLHLFPIDLQCASAQQIAAAHMQNLPRLVRGALRRMGLGRVSKEIVFEYMPELFEPSRIAYFHGYFQDPRYFEDISPLIKQTFTLPHPTEHAEQYSRKLSQILAAKNSVFVHIRRGDYMRLGWQLDISYQLRAIAYMAKRVQNLELFLFCEDLEFVQNLDLGYPFVDMTTRDGAAHWDMMLMQSCKHGIITNSTYSWWAAYLIKNPEKIIIGPSHWIYGNENILCKDWVKIESQFETKS

SEQ ID NO: 9 - DNA, 903 bp, Helicobacter pylori 26695
  source 1..903: mol_type = genomic DNA
atggcttttaaggtggtgcaaatttgcggagggcttgggaatcaaatgtttcaatacgctttcgctaaaagtttgcaaaaacactctaatacgcctgtgctgttagatatcacttcttttgattggagcgataggaaaatgcaattagaacttttccctattgatttgccctatgcgagcgcgaaagaaatcgctatagctaaaatgcaacacctccccaagctagtaagagacgcgctcaaatgcatgggatttgatagggtgagtcaagaaatcgtttttgaatacgagcctaaattgctaaagccaagccgcttgacttatttttttggctatttccaagatccacgatactttgatgctatatcccctttaatcaagcaaaccttcactctaccaccaccaccagaaaataataagaataataataaaaaagaggaagaatatcagtgcaagctttctttgattttagccgctaaaaacagcgtgtttgtgcatataagaagaggggattatgtggggattggctgtcagcttggtattgactatcaaaaaaaggcgcttgagtatatggcaaagcgcgtgccaaacatggagctttttgtgttttgcgaagacttagaattcacgcaaaatcttgatcttggctacccttttatggacatgaccactagggataaagaagaagaggcgtattgggacatgctgctcatgcaatcttgtcagcatggcattatcgctaatagcacttatagctggtgggcggcctatttgatagaaaatccagaaaaaatcattattggccccaaacactggctttttgggcatgagaatatcctttgtaaggagtgggtgaaaatagaatcccattttgaggtaaaatcccaaaagtataacgcttaa

SEQ ID NO: 10 - protein, 300 aa, Helicobacter pylori 26695
MAFKVVQICGGLGNQMFQYAFAKSLQKHSNTPVLLDITSFDWSDRKMQLELFPIDLPYASAKEIAIAKMQHLPKLVRDALKCMGFDRVSQEIVFEYEPKLLKPSRLTYFFGYFQDPRYFDAISPLIKQTFTLPPPPENNKNNNKKEEEYQCKLSLILAAKNSVFVHIRRGDYVGIGCQLGIDYQKKALEYMAKRVPNMELFVFCEDLEFTQNLDLGYPFMDMTTRDKEEEAYWDMLLMQSCQHGIIANSTYSWWAAYLIENPEKIIIGPKHWLFGHENILCKEWVKIESHFEVKSQKYNA

SEQ ID NO: 11 - DNA, 882 bp, Thermosynechococcus elongatus BP-1
  source 1..882: mol_type = genomic DNA
atgattatcgttcacctgtgcggcggcctgggcaaccaaatgtttcaatacgcggcgggtctggcggcggcgcatcgcatcggcagcgaggtgaagttcgatacccactggtttgacgcgacctgcctgcaccaaggtctggagctgcgtcgtgtgtttggtctggaactgccggaaccgagcagcaaggatctgcgtaaggttctgggtgcgtgcgttcacccggcggttcgtcgtctgctggcgggtcactttctgcacggtctgcgtccgaaaagcctggtgatccaaccgcactttcactactggaccggttttgagcacctgccggataacgtgtacctggaaggttactggcaaagcgaacgttacttcagcaacatcgcggacattatccgtcagcaattccgttttgtggaaccgctggacccgcacaacgcggcgctgatggacgagatgcaaagcggtgtgagcgttagcctgcacattcgtcgtggtgactacttcaacaacccgcaaatgcgtcgtgttcacggtgttgatctgagcgaatactatccggcggcggttgcgaccatgatcgagaagaccaacgcggaacgtttttacgtgttcagcgatgacccgcaatgggttctggaacacctgaaactgccggttagctataccgtggttgatcacaaccgtggtgcggcgagctatcgtgacatgcaactgatgagcgcgtgccgtcaccacatcattgcgaacagcacctttagctggtggggtgcgtggctgaacccgcgtccggataaggtggttattgcgccgcgtcactggtttaatgttgatgtttttgacacccgtgacctgtattgcccgggttggattgttctgtaa

SEQ ID NO: 12 - protein, 293 aa, Thermosynechococcus elongatus BP-1
MIIVHLCGGLGNQMFQYAAGLAAAHRIGSEVKFDTHWFDATCLHQGLELRRVFGLELPEPSSKDLRKVLGACVHPAVRRLLAGHFLHGLRPKSLVIQPHFHYWTGFEHLPDNVYLEGYWQSERYFSNIADIIRQQFRFVEPLDPHNAALMDEMQSGVSVSLHIRRGDYFNNPQMRRVHGVDLSEYYPAAVATMIEKTNAERFYVFSDDPQWVLEHLKLPVSYTVVDHNRGAASYRDMQLMSACRHHIIANSTFSWWGAWLNPRPDKVVIAPRHWFNVDVFDTRDLYCPGWIVL

SEQ ID NO: 13 - DNA, 1233 bp, E. coli W3110
  source 1..1233: mol_type = genomic DNA
atgcaaaataaattagcttccggtgccaggcttggacgtcaggcgttacttttccctctctgtctggtgctttacgaattttcaacctatatcggcaacgatatgattcaacccggtatgttggccgtggtggaacaatatcaggcgggcattgattgggttcctacttcgatgaccgcgtatctggcgggcgggatgtttttacaatggctgctggggccgctgtcggatcgtattggtcgccgtccggtgatgctggcgggagtggtgtggtttatcgtcacctgtctggcaatattgctggcgcaaaacattgaacaattcaccctgttgcgcttcttgcagggcataagcctctgtttcattggcgctgtgggatacgccgcaattcaggaatccttcgaagaggcggtttgtatcaagatcaccgcgctgatggcgaacgtggcgctgattgctccgctacttggtccgctggtgggcgcggcgtggatccatgtgctgccctgggaggggatgtttgttttgtttgccgcattggcagcgatctcctttttcggtctgcaacgagccatgcctgaaaccgccacgcgtataggcgagaaactgtcactgaaagaactcggtcgtgactataagctggtgctgaagaacggccgctttgtggcgggggcgctggcgctgggattcgttagtctgccgttgctggcgtggatcgcccagtcgccgattatcatcattaccggcgagcagttgagcagctatgaatatggcttgctgcaagtgcctattttcggggcgttaattgcgggtaacttgctgttagcgcgtctgacctcgcgccgcaccgtacgttcgctgattattatgggcggctggccgattatgattggtctattggtcgctgctgcggcaacggttatctcatcgcacgcgtatttatggatgactgccgggttaagtatttatgctttcggtattggtctggcgaatgcgggactggtgcgattaaccctgtttgccagcgatatgagtaaaggtacggtttctgccgcgatgggaatgctgcaaatgctgatctttaccgttggtattgaaatcagcaaacatgcctggctgaacgggggcaacggactgtttaatctcttcaaccttgtcaacggaattttgtggctgtcgctgatggttatctttttaaaagataaacagatgggaaattctcacgaagggtaa

SEQ ID NO: 14 - protein, 410 aa, E. coli W3110
MQNKLASGARLGRQALLFPLCLVLYEFSTYIGNDMIQPGMLAVVEQYQAGIDWVPTSMTAYLAGGMFLQWLLGPLSDRIGRRPVMLAGVVWFIVTCLAILLAQNIEQFTLLRFLQGISLCFIGAVGYAAIQESFEEAVCIKITALMANVALIAPLLGPLVGAAWIHVLPWEGMFVLFAALAAISFFGLQRAMPETATRIGEKLSLKELGRDYKLVLKNGRFVAGALALGFVSLPLLAWIAQSPIIIITGEQLSSYEYGLLQVPIFGALIAGNLLLARLTSRRTVRSLIIMGGWPIMIGLLVAAAATVISSHAYLWMTAGLSIYAFGIGLANAGLVRLTLFASDMSKGTVSAAMGMLQMLIFTVGIEISKHAWLNGGNGLFNLFNLVNGILWLSLMVIFLKDKQMGNSHEG

SEQ ID NO: 15 - DNA, 20 bp, synthetic construct
  misc_feature 1..20: note = Description of the artificial sequence: base sequence foramplification ofcatsacB fragment
  source 1..20: mol_type = other DNA
accaggcgtttaagggcacc

SEQ ID NO: 16 - DNA, 21 bp, synthetic construct
  misc_feature 1..21: note = Description of the artificial sequence: base sequence foramplification of catsacB fragment
  source 1..21: mol_type = other DNA
tacggttagccatttgcctgc

SEQ ID NO: 17 - DNA, 42 bp, synthetic construct
  misc_feature 1..42: note = Description of the artificial sequence: base sequence foramplification of lacZ upstream 1 fragment
  source 1..42: mol_type = other DNA
ggtgcccttaaacgcctggtagctgtttcctgtgtgaaattg

SEQ ID NO: 18 - DNA, 18 bp, synthetic construct
  misc_feature 1..18: note = Description of the artificial sequence: base sequence foramplification of lacZ upstream 1 fragment
  source 1..18: mol_type = other DNA
ccagtctggccctgcacg

SEQ ID NO: 19 - DNA, 43 bp, synthetic construct
  misc_feature 1..43: note = Description of the artificial sequence: base sequence foramplification of lacY downstream 1 fragment
  source 1..43: mol_type = other DNA
gcaggcaaatggctaaccgtacgaccaacatatcataacggag

SEQ ID NO: 20 - DNA, 20 bp, synthetic construct
  misc_feature 1..20: note = Description of the artificial sequence: base sequence foramplification of lacY downstream 1 fragment
  source 1..20: mol_type = other DNA
gtttccgctctgtttgctgc

SEQ ID NO: 21 - DNA, 42 bp, synthetic construct
  misc_feature 1..42: note = Description of the artificial sequence: base sequence foramplification of lacZ upstream 2 fragment
  source 1..42: mol_type = other DNA
ccgttatgatatgttggtcgagctgtttcctgtgtgaaattg

SEQ ID NO: 22 - DNA, 22 bp, synthetic construct
  misc_feature 1..22: note = Description of the artificial sequence: base sequence foramplification of lacY downstream 2 fragment
  source 1..22: mol_type = other DNA
cgaccaacatatcataacggag

SEQ ID NO: 23 - DNA, 41 bp, synthetic construct
  misc_feature 1..41: note = Description of the artificial sequence: base sequence foramplification of wcaJ upstream 1 fragment
  source 1..41: mol_type = other DNA
ggtgcccttaaacgcctggtcgttgttcctgttattagccc

SEQ ID NO: 24 - DNA, 20 bp, synthetic construct
  misc_feature 1..20: note = Description of the artificial sequence: base sequence foramplification of wcaJ upstream 1fragment
  source 1..20: mol_type = other DNA
acgcggtcgctatcagcaaa

SEQ ID NO: 25 - DNA, 44 bp, synthetic construct
  misc_feature 1..44: note = Description of the artificial sequence: base sequence foramplification of wcaM downstream 1 fragment
  source 1..44: mol_type = other DNA
gcaggcaaatggctaaccgtaatttgcgaccattcctggaaaaa

SEQ ID NO: 26 - DNA, 23 bp, synthetic construct
  misc_feature 1..23: note = Description of the artificial sequence: base sequence foramplification of wcaM downstream 1 fragment
  source 1..23: mol_type = other DNA
acttcacaaacgcctgcatatag

SEQ ID NO: 27 - DNA, 41 bp, synthetic construct
  misc_feature 1..41: note = Description of the artificial sequence: base sequence foramplification of wcaJ upstream 2 fragment
  source 1..41: mol_type = other DNA
ttccaggaatggtcgcaaatcgttgttcctgttattagccc

SEQ ID NO: 28 - DNA, 23 bp, synthetic construct
  misc_feature 1..23: note = Description of the artificial sequence: base sequence foramplification of wcaM downstream 2 fragment
  source 1..23: mol_type = other DNA
atttgcgaccattcctggaaaaa

SEQ ID NO: 29 - DNA, 20 bp, synthetic construct
  misc_feature 1..20: note = Description of the artificial sequence: base sequence foramplification of pMW118 fragment
  source 1..20: mol_type = other DNA
agctgtttcctgtgtgaaat

SEQ ID NO: 30 - DNA, 18 bp, synthetic construct
  misc_feature 1..18: note = Description of the artificial sequence: base sequence foramplification of pMW118 fragment
  source 1..18: mol_type = other DNA
accctggcgttacccaac

SEQ ID NO: 31 - DNA, 39 bp, synthetic construct
  misc_feature 1..39: note = Description of the artificial sequence: base sequence foramplification of mdfA fragment
  source 1..39: mol_type = other DNA
acacaggaaacagctatgcaaaataaattagcttccggt

SEQ ID NO: 32 - DNA, 36 bp, synthetic construct
  misc_feature 1..36: note = Description of the artificial sequence: base sequence foramplification of mdfA fragment
  source 1..36: mol_type = other DNA
gggtaacgccagggtttacccttcgtgagaatttcc

SEQ ID NO: 33 - DNA, 24 bp, synthetic construct
  misc_feature 1..24: note = Description of the artificial sequence: base sequence foramplification of pUAKQE fragment
  source 1..24: mol_type = other DNA
ggttaatttctcctctttaatatc

SEQ ID NO: 34 - DNA, 22 bp, synthetic construct
  misc_feature 1..22: note = Description of the artificial sequence: base sequence foramplification of pUAKQE fragment
  source 1..22: mol_type = other DNA
catcaccatcaccatcactaag

SEQ ID NO: 35 - DNA, 36 bp, synthetic construct
  misc_feature 1..36: note = Description of the artificial sequence: base sequence foramplification of rcsA fragment
  source 1..36: mol_type = other DNA
gaggagaaattaaccgcattgagtgagggtatgcca

SEQ ID NO: 36 - DNA, 44 bp, synthetic construct
  misc_feature 1..44: note = Description of the artificial sequence: base sequence foramplification of rcsA fragment
  source 1..44: mol_type = other DNA
aatggatttccttacgcgaattagcgcatgttgacaaaaatacc

SEQ ID NO: 37 - DNA, 23 bp, synthetic construct
  misc_feature 1..23: note = Description of the artificial sequence: base sequence foramplification of lacY fragment
  source 1..23: mol_type = other DNA
ttcgcgtaaggaaatccattatg

SEQ ID NO: 38 - DNA, 38 bp, synthetic construct
  misc_feature 1..38: note = Description of the artificial sequence: base sequence foramplification of lacY fragment
  source 1..38: mol_type = other DNA
atggtgatggtgatgttaagcgacttcattcacctgac

SEQ ID NO: 39 - DNA, 21 bp, synthetic construct
  misc_feature 1..21: note = Description of the artificial sequence: base sequence foramplification of pUAKQE-rcsA-lacY fragment
  source 1..21: mol_type = other DNA
gcattgagtgagggtatgcca

SEQ ID NO: 40 - DNA, 43 bp, synthetic construct
  misc_feature 1..43: note = Description of the artificial sequence: base sequence foramplification of HMFT fragment
  source 1..43: mol_type = other DNA
gatattaaagaggagaaattaaccatggattttaagattgtgc

SEQ ID NO: 41 - DNA, 41 bp, synthetic construct
  misc_feature 1..41: note = Description of the artificial sequence: base sequence foramplification of HMFT fragment
  source 1..41: mol_type = other DNA
ggcataccctcactcaatgctcaagattttgtctcaaattg

SEQ ID NO: 42 - DNA, 44 bp, synthetic construct
  misc_feature 1..44: note = Description of the artificial sequence: base sequence foramplification of FutC fragment
  source 1..44: mol_type = other DNA
gatattaaagaggagaaattaaccatggcttttaaggtggtgca

SEQ ID NO: 43 - DNA, 38 bp, synthetic construct
  misc_feature 1..38: note = Description of the artificial sequence: base sequence foramplification of FutC fragment
  source 1..38: mol_type = other DNA
ggcataccctcactcaatgcttaagcgttatacttttg

SEQ ID NO: 44 - DNA, 46 bp, synthetic construct
  misc_feature 1..46: note = Description of the artificial sequence: base sequence foramplification of Te2FT fragment
  source 1..46: mol_type = other DNA
gatattaaagaggagaaattaaccatgattatcgttcacctgtgcg

SEQ ID NO: 45 - DNA, 38 bp, synthetic construct
  misc_feature 1..38: note = Description of the artificial sequence: base sequence foramplification of Te2FT fragment
  source 1..38: mol_type = other DNA
ggcataccctcactcaatgcttacagaacaatccaacc

SEQ ID NO: 46 - DNA, 40 bp, synthetic construct
  misc_feature 1..40: note = Description of the artificial sequence: base sequence foramplification of BffucT fragment
  source 1..40: mol_type = other DNA
gaggagaaattaaccatgtgtgattgcttgtctatcatat

SEQ ID NO: 47 - DNA, 40 bp, synthetic construct
  misc_feature 1..40: note = Description of the artificial sequence: base sequence foramplification of BffucT fragment
  source 1..40: mol_type = other DNA
accctcactcaatgcttattttctatcaaacaattgagaa

SEQ ID NO: 48 - DNA, 37 bp, synthetic construct
  misc_feature 1..37: note = Description of the artificial sequence: base sequence foramplification of HpfutA fragment
  source 1..37: mol_type = other DNA
gaggagaaattaaccatgttccaacccctattagacg

SEQ ID NO: 49 - DNA, 40 bp, synthetic construct
  misc_feature 1..40: note = Description of the artificial sequence: base sequence foramplification of HpfutA fragment
  source 1..40: mol_type = other DNA
accctcactcaatgcttacaaacccaattttttaaccaac

SEQ ID NO: 50 - DNA, 40 bp, synthetic construct
  misc_feature 1..40: note = Description of the artificial sequence: base sequence foramplification of cBrfucT Upstream fragment
  source 1..40: mol_type = other DNA
gaggagaaattaaccatgaaattgaaagtgaaatttgtag

SEQ ID NO: 51 - DNA, 22 bp, synthetic construct
  misc_feature 1..22: note = Description of the artificial sequence: base sequence foramplification ofcBrfucT Upstreamfragment
  source 1..22: mol_type = other DNA
attcagagcttcctgtgaatta

SEQ ID NO: 52 - DNA, 41 bp, synthetic construct
  misc_feature 1..41: note = Description of the artificial sequence: base sequence foramplification of cBrfucT midstream fragment
  source 1..41: mol_type = other DNA
attcacaggaagctctgaatcgtaagttctgcagcatcgtg

SEQ ID NO: 53 - DNA, 20 bp, synthetic construct
  misc_feature 1..20: note = Description of the artificial sequence: base sequence foramplification of cBrfucT midstream fragment
  source 1..20: mol_type = other DNA
accccagtaaaccggaatgc

SEQ ID NO: 54 - DNA, 40 bp, synthetic construct
  misc_feature 1..40: note = Description of the artificial sequence: base sequence foramplification of cBrfucT downstream fragment
  source 1..40: mol_type = other DNA
gcattccggtttactggggtaacagattggttgagttgga

SEQ ID NO: 55 - DNA, 38 bp, synthetic construct
  misc_feature 1..38: note = Description of the artificial sequence: base sequence foramplification of cBrfucT downstream fragment
  source 1..38: mol_type = other DNA
accctcactcaatgctcatctaaaccaacgacaagggt

SEQ ID NO: 56 - DNA, 63 bp, synthetic construct
  misc_feature 1..63: note = Description of the artificial sequence: base sequence foramplification offragment
  source 1..63: mol_type = other DNA
tgcacaatcttaaaatccatggttaatttctcctctttaattcatctaaaccaacgacaaggg

SEQ ID NO: 57 - DNA, 24 bp, synthetic construct
  misc_feature 1..24: note = Description of the artificial sequence: base sequence foramplification of HMFT fragment
  source 1..24: mol_type = other DNA
atggattttaagattgtgcaagtg

SEQ ID NO: 58 - DNA, 61 bp, synthetic construct
  misc_feature 1..61: note = Description of the artificial sequence: base sequence foramplification of BffucT fragment
  source 1..61: mol_type = other DNA
aatcttaaaatccatggttaatttctcctctttaatttattttctatcaaacaattgagaa

SEQ ID NO: 59 - DNA, 61 bp, synthetic construct
  misc_feature 1..61: note = Description of the artificial sequence: base sequence foramplification of HpfutA fragment
  source 1..61: mol_type = other DNA
aatcttaaaatccatggttaatttctcctctttaatttacaaacccaattttttaaccaac

SEQ ID NO: 60 - DNA, 43 bp, synthetic construct
  misc_feature 1..43: note = Description of the artificial sequence: base sequence foramplification of cBrfucT fragment
  source 1..43: mol_type = other DNA
ggttaatttctcctctttaattcatctaaaccaacgacaaggg

SEQ ID NO: 61 - DNA, 39 bp, synthetic construct
  misc_feature 1..39: note = Description of the artificial sequence: base sequence foramplification of futC fragment
  source 1..39: mol_type = other DNA
gaggagaaattaaccatggcttttaaggtggtgcaaatt

SEQ ID NO: 62 - DNA, 43 bp, synthetic construct; identical to SEQ ID NO: 60
  misc_feature 1..43: note = Description of the artificial sequence: base sequence foramplification of cBrfucT fragment
  source 1..43: mol_type = other DNA

SEQ ID NO: 63 - DNA, 38 bp, synthetic construct
  misc_feature 1..38: note = Description of the artificial sequence: base sequence foramplification of cBrfucT fragment
  source 1..38: mol_type = other DNA
gaggagaaattaaccatgattatcgttcacctgtgcgg

SEQ ID NO: 64 - DNA, 264 bp, synthetic construct
  misc_feature 1..264: note = Description of the artificial sequence: base sequence of partialsequence of codon-optimised BfFucT
  source 1..264: mol_type = other DNA
cgtaagttctgcagcatcgtggttagcaataataaatgggcggacccgattcgtgagacctttttcaaactgctgagcagctacaaaaaggtggacagcggtggccgtgcgtggaacaacatcggtggcccggttgacaacaagctggatttcatcagccagtacaaattcaacattgcgtttgagaacagccgtgtgctgggttacaccaccgaaaagattatggagccgatgcaagtgaacagcattccggtttactggggt